European Patent Specification EP 3 504 231 B1, published February 4, 2026. Title: Promoter for Cell-Specific Gene Expression and Uses thereof. Applicant: Università del Piemonte Orientale. The sequence listing filed with the application follows.

SEQUENCE LISTING (30 sequences)

SEQ ID NO: 1 - DNA, 1175 bp, Artificial Sequence
  LV.pF8.1
gagctcaccatggctacattctgatgtaaagagatatatcctatacctgggccaaatgtaaacagcctggaaaagtgttaggttaaaaacaaaacaaaataaataaatgaataaatgccaggtggttatgagtgctattgagaaaaatgaagccaagagggatatcagtgatgcaggtgggggtaaagagcttacaacataaatgtggtgttccatatttaaacctcattcaacagggaagattggagctgaaatgtgaaggagttgtgggagtggaactacgtggaaatctgggggaaaggtgttttgggtaaaagaaatagcaagtgttgaggtccaggggcatgagtgtgcttgatattttagggaagagtaaggagaccagtataaccagagtgagatgagactacagaggtcaggagaaagggcatgcagaccatgtgggatgctctaggacctaggccatggtaaagatgtagggttttaccctgatggaggtcagaagccattggaggattctgagaagaggagtgacaggactcgctttatagttttaaattataactataaattatagtttttaaaacaatagttgcctaacctcatgttatatgtaaaactacagttttaaaaactataaattcctcatactggcagcagtgtgaggggcaagggcaaaagcagagagactaacaggttgctggttactcttgctagtgcaagtgaattctagaatcttcgacaacatccagaacttctcttgctgctgccactcaggaagagggttggagtaggctaggaataggagcacaaattaaagctcctgttcactttgacttctccatccctctcctcctttccttaaaggttctgattaaagcagacttatgcccctactgctctcagaagtgaatgggttaagtttagcagcctcccttttgctacttcagttcttcctgtggctgcttcccactgataaaaaggaagcaatcctatcggttactgcttagtgctgagcacatccagtgggtaaagttccttaaaatgctctgcaaagaaattgggacttttcattaaatcagaaattttacttttttcccctcctgggagctaaagatattttagagaagaattaaccttttgcttctccagttgaacatttgtagcaataagtc

SEQ ID NO: 2 - DNA, 599 bp, Artificial Sequence
  LV.pF8.2
gtttttaaaacaatagttgcctaacctcatgttatatgtaaaactacagttttaaaaactataaattcctcatactggcagcagtgtgaggggcaagggcaaaagcagagagactaacaggttgctggttactcttgctagtgcaagtgaattctagaatcttcgacaacatccagaacttctcttgctgctgccactcaggaagagggttggagtaggctaggaataggagcacaaattaaagctcctgttcactttgacttctccatccctctcctcctttccttaaaggttctgattaaagcagacttatgcccctactgctctcagaagtgaatgggttaagtttagcagcctcccttttgctacttcagttcttcctgtggctgcttcccactgataaaaaggaagcaatcctatcggttactgcttagtgctgagcacatccagtgggtaaagttccttaaaatgctctgcaaagaaattgggacttttcattaaatcagaaattttacttttttcccctcctgggagctaaagatattttagagaagaattaaccttttgcttctccagttgaacatttgtagcaataagtc

SEQ ID NO: 3 - DNA, 1698 bp, Artificial Sequence
  LV.pF8.3
ggggctcgctcgctcagtacctggaggcgagttcctgacgcgactgcgactcaatcctcgcctggtgaagaatattttacctatgactcactgaaaataaagacggctgagtgaccgtgtttgttcatgtaaacattgaacaaatatttatcggcttctgcgatgtgtcctactcttttagtggaggaagacacattttatttatgtatttaatttttcttttgaattttacatgcgagttatacttaataaaactcacttcaaaatataccttcaacagaaaatccagcaacagtttctattatgttagttaaaacagccagtcttttcctttacttttaaaaattattcataaatgtaattagtgaatgataataaacattgacatctgatccactgctttaggagtgacacaaatgaagttaactcaggctattttctttataatcattgtgctattgttttctttttcttttcaattatactgcttaatataggattttgtggcaccataggagttgaggagctcaccatggctacattctgatgtaaagagatatatcctatacctgggccaaatgtaaacagcctggaaaagtgttaggttaaaaacaaaacaaaataaataaatgaataaatgccaggtggttatgagtgctattgagaaaaatgaagccaagagggatatcagtgatgcaggtgggggtaaagagcttacaacataaatgtggtgttccatatttaaacctcattcaacagggaagattggagctgaaatgtgaaggagttgtgggagtggaactacgtggaaatctgggggaaaggtgttttgggtaaaagaaatagcaagtgttgaggtccaggggcatgagtgtgcttgatattttagggaagagtaaggagaccagtataaccagagtgagatgagactacagaggtcaggagaaagggcatgcagaccatgtgggatgctctaggacctaggccatggtaaagatgtagggttttaccctgatggaggtcagaagccattggaggattctgagaagaggagtgacaggactcgctttatagttttaaattataactataaattatagtttttaaaacaatagttgcctaacctcatgttatatgtaaaactacagttttaaaaactataaattcctcatactggcagcagtgtgaggggcaagggcaaaagcagagagactaacaggttgctggttactcttgctagtgcaagtgaattctagaatcttcgacaacatccagaacttctcttgctgctgccactcaggaagagggttggagtaggctaggaataggagcacaaattaaagctcctgttcactttgacttctccatccctctcctcctttccttaaaggttctgattaaagcagacttatgcccctactgctctcagaagtgaatgggttaagtttagcagcctcccttttgctacttcagttcttcctgtggctgcttcccactgataaaaaggaagcaatcctatcggttactgcttagtgctgagcacatccagtgggtaaagttccttaaaatgctctgcaaagaaattgggacttttcattaaatcagaaattttacttttttcccctcctgggagctaaagatattttagagaagaattaaccttttgcttctccagttgaacatttgtagcaataagtc

SEQ ID NO: 4 - DNA, 1122 bp, Artificial Sequence
  LV.pF8.4
ggggctcgctcgctcagtacctggaggcgagttcctgacgcgactgcgactcaatcctcgcctggtgaagaatattttacctatgactcactgaaaataaagacggctgagtgaccgtgtttgttcatgtaaacattgaacaaatatttatcggcttctgcgatgtgtcctactcttttagtggaggaagacacattttatttatgtatttaatttttcttttgaattttacatgcgagttatacttaataaaactcacttcaaaatataccttcaacagaaaatccagcaacagtttctattatgttagttaaaacagccagtcttttcctttacttttaaaaattattcataaatgtaattagtgaatgataataaacattgacatctgatccactgctttaggagtgacacaaatgaagttaactcaggctattttctttataatcattgtgctattgttttctttttcttttcaattatactgcttaatataggattttgtggcaccataggagttgaggtttttaaaacaatagttgcctaacctcatgttatatgtaaaactacagttttaaaaactataaattcctcatactggcagcagtgtgaggggcaagggcaaaagcagagagactaacaggttgctggttactcttgctagtgcaagtgaattctagaatcttcgacaacatccagaacttctcttgctgctgccactcaggaagagggttggagtaggctaggaataggagcacaaattaaagctcctgttcactttgacttctccatccctctcctcctttccttaaaggttctgattaaagcagacttatgcccctactgctctcagaagtgaatgggttaagtttagcagcctcccttttgctacttcagttcttcctgtggctgcttcccactgataaaaaggaagcaatcctatcggttactgcttagtgctgagcacatccagtgggtaaagttccttaaaatgctctgcaaagaaattgggacttttcattaaatcagaaattttacttttttcccctcctgggagctaaagatattttagagaagaattaaccttttgcttctccagttgaacatttgtagcaataagtc

SEQ ID NO: 5 - DNA, 1979 bp, Artificial Sequence
  LV.pF8.5
tcgccaccacttggcttccggcacgtggggcagatgtttccattcccacggcggcagcggaagagggagggccgggcgcgccgcggctgcttgcagtctccgcaagcggctacatcacagagctcagcgtgcggtgtcacaggccccgcggtcccgcccaacagatgcaccgagatgcgcgtgcgcagaaagcgtcccgggggtgaggctccctccctcgctctccctctactcccgccccactctcccccactttcccccctccacccaccgcggccgtcggggctcgctcgctcagtacctggaggcgagttcctgacgcgactgcgactcaatcctcgcctggtgaagaatattttacctatgactcactgaaaataaagacggctgagtgaccgtgtttgttcatgtaaacattgaacaaatatttatcggcttctgcgatgtgtcctactcttttagtggaggaagacacattttatttatgtatttaatttttcttttgaattttacatgcgagttatacttaataaaactcacttcaaaatataccttcaacagaaaatccagcaacagtttctattatgttagttaaaacagccagtcttttcctttacttttaaaaattattcataaatgtaattagtgaatgataataaacattgacatctgatccactgctttaggagtgacacaaatgaagttaactcaggctattttctttataatcattgtgctattgttttctttttcttttcaattatactgcttaatataggattttgtggcaccataggagttgaggagctcaccatggctacattctgatgtaaagagatatatcctatacctgggccaaatgtaaacagcctggaaaagtgttaggttaaaaacaaaacaaaataaataaatgaataaatgccaggtggttatgagtgctattgagaaaaatgaagccaagagggatatcagtgatgcaggtgggggtaaagagcttacaacataaatgtggtgttccatatttaaacctcattcaacagggaagattggagctgaaatgtgaaggagttgtgggagtggaactacgtggaaatctgggggaaaggtgttttgggtaaaagaaatagcaagtgttgaggtccaggggcatgagtgtgcttgatattttagggaagagtaaggagaccagtataaccagagtgagatgagactacagaggtcaggagaaagggcatgcagaccatgtgggatgctctaggacctaggccatggtaaagatgtagggttttaccctgatggaggtcagaagccattggaggattctgagaagaggagtgacaggactcgctttatagttttaaattataactataaattatagtttttaaaacaatagttgcctaacctcatgttatatgtaaaactacagttttaaaaactataaattcctcatactggcagcagtgtgaggggcaagggcaaaagcagagagactaacaggttgctggttactcttgctagtgcaagtgaattctagaatcttcgacaacatccagaacttctcttgctgctgccactcaggaagagggttggagtaggctaggaataggagcacaaattaaagctcctgttcactttgacttctccatccctctcctcctttccttaaaggttctgattaaagcagacttatgcccctactgctctcagaagtgaatgggttaagtttagcagcctcccttttgctacttcagttcttcctgtggctgcttcccactgataaaaaggaagcaatcctatcggttactgcttagtgctgagcacatccagtgggtaaagttccttaaaatgctctgcaaagaaattgggacttttcattaaatcagaaattttacttttttcccctcctgggagctaaagatattttagagaagaattaaccttttgcttctccagttgaacatttgtagcaataagtc

SEQ ID NO: 6 - DNA, 1403 bp, Artificial Sequence
  LV.pF8.6
tcgccaccacttggcttccggcacgtggggcagatgtttccattcccacggcggcagcggaagagggagggccgggcgcgccgcggctgcttgcagtctccgcaagcggctacatcacagagctcagcgtgcggtgtcacaggccccgcggtcccgcccaacagatgcaccgagatgcgcgtgcgcagaaagcgtcccgggggtgaggctccctccctcgctctccctctactcccgccccactctcccccactttcccccctccacccaccgcggccgtcggggctcgctcgctcagtacctggaggcgagttcctgacgcgactgcgactcaatcctcgcctggtgaagaatattttacctatgactcactgaaaataaagacggctgagtgaccgtgtttgttcatgtaaacattgaacaaatatttatcggcttctgcgatgtgtcctactcttttagtggaggaagacacattttatttatgtatttaatttttcttttgaattttacatgcgagttatacttaataaaactcacttcaaaatataccttcaacagaaaatccagcaacagtttctattatgttagttaaaacagccagtcttttcctttacttttaaaaattattcataaatgtaattagtgaatgataataaacattgacatctgatccactgctttaggagtgacacaaatgaagttaactcaggctattttctttataatcattgtgctattgttttctttttcttttcaattatactgcttaatataggattttgtggcaccataggagttgaggtttttaaaacaatagttgcctaacctcatgttatatgtaaaactacagttttaaaaactataaattcctcatactggcagcagtgtgaggggcaagggcaaaagcagagagactaacaggttgctggttactcttgctagtgcaagtgaattctagaatcttcgacaacatccagaacttctcttgctgctgccactcaggaagagggttggagtaggctaggaataggagcacaaattaaagctcctgttcactttgacttctccatccctctcctcctttccttaaaggttctgattaaagcagacttatgcccctactgctctcagaagtgaatgggttaagtttagcagcctcccttttgctacttcagttcttcctgtggctgcttcccactgataaaaaggaagcaatcctatcggttactgcttagtgctgagcacatccagtgggtaaagttccttaaaatgctctgcaaagaaattgggacttttcattaaatcagaaattttacttttttcccctcctgggagctaaagatattttagagaagaattaaccttttgcttctccagttgaacatttgtagcaataagtc

SEQ ID NO: 7 - DNA, 2350 bp, Artificial Sequence
  0 to 2350 5' FVIII promoter sequence
cagcagttcccacaaacgttaccctcacaatgaatccagccatttttcaccctctccagtggtaccatcatagcccaagccgccaccatttctcacccccggttaacaggccaccctccttctacccttatcctgctagagtttgttttatctacagtgatcagaaagatcagcctaaaagataattctgatcaccaccctcctctactcacaacccggccgtgtctccccattgccctcagtgtagaagtcaatgtccctttgctgaaatgcaaccttagtgaaactttccatgactaacctcctttaaaattgcaacctggtccacccttactcccccttaccccacttctcttttttgcacagcacttattttaccttctaacatactgtataatgtactcatgtattgtaattattgcttatcatccctctttcagttgcttatatttttcatcaatgtgtacccagtgcctaggacaatatctgtctaggacaaatgggtagttatgtggctgtaggcaagccatttaacctctctgtacctcagttactttatctgtatccactttgcggtgttgtcatgaggattaaatcagatagcctatgtgtagcacctggcagtgaatttatcaccctgtactgtaactgtctacttttctgtctcctccattggactgtcattcccagggggttgggaactgggatttcttcatttctgaggcatagaagtatagcatagtggttaggagcatgacttctggagccagagtacatgggtttgaatgctaccactcacaagctgtgtggccatggagaagttgcctaacctctccgtgcttcagtttcatcacccataaaatgaaggtaagaatagtacctgtatttaaaagcacctagaacagttcctggcatatagtgtcagctgtcatctctgcatccttgtacctgtcagagaggagtgtttatcaaaggggcttcttgctgcctgtttccaaaccagtcgacaatataccaattgctccctaacacattcttgtttgtgcagaactgagctcaatgataacatttttatagcaaccctgatcaagtttcttctcataatctcttacactttgaggcccctgcaggggccctcactctccctaataaacattaacctgagtagggtgtttgagctcaccatggctacattctgatgtaaagagatatatcctatacctgggccaaatgtaaacagcctggaaaagtgttaggttaaaaacaaaacaaaataaataaatgaataaatgccaggtggttatgagtgctattgagaaaaatgaagccaagagggatatcagtgatgcaggtgggggtaaagagcttacaacataaatgtggtgttccatatttaaacctcattcaacagggaagattggagctgaaatgtgaaggagttgtgggagtggaactacgtggaaatctgggggaaaggtgttttgggtaaaagaaatagcaagtgttgaggtccaggggcatgagtgtgcttgatattttagggaagagtaaggagaccagtataaccagagtgagatgagactacagaggtcaggagaaagggcatgcagaccatgtgggatgctctaggacctaggccatggtaaagatgtagggttttaccctgatggaggtcagaagccattggaggattctgagaagaggagtgacaggactcgctttatagttttaaattataactataaattatagtttttaaaacaatagttgcctaacctcatgttatatgtaaaactacagttttaaaaactataaattcctcatactggcagcagtgtgaggggcaagggcaaaagcagagagactaacaggttgctggttactcttgctagtgcaagtgaattctagaatcttcgacaacatccagaacttctcttgctgctgccactcaggaagagggttggagtaggctaggaataggagcacaaattaaagctcctgttcactttgacttctccatccctctcctcctttccttaaaggttctgattaaagcagacttatgcccctactgctctcagaagtgaatgggttaagtttagcagcctcccttttgctacttcagttcttcctgtggctgcttcccactgataaaaaggaagcaatcctatcggttactgcttagtgctgagcacatccagtgggtaaagttccttaaaatgctctgcaaagaaattgggacttttcattaaatcagaaattttacttttttcccctcctgggagctaaagatattttagagaagaattaaccttttgcttctccagttgaacatttgtagcaataagtc

SEQ ID NO: 8 - DNA, 523 bp, Artificial Sequence
  Enhancer Short
ggggctcgctcgctcagtacctggaggcgagttcctgacgcgactgcgactcaatcctcgcctggtgaagaatattttacctatgactcactgaaaataaagacggctgagtgaccgtgtttgttcatgtaaacattgaacaaatatttatcggcttctgcgatgtgtcctactcttttagtggaggaagacacattttatttatgtatttaatttttcttttgaattttacatgcgagttatacttaataaaactcacttcaaaatataccttcaacagaaaatccagcaacagtttctattatgttagttaaaacagccagtcttttcctttacttttaaaaattattcataaatgtaattagtgaatgataataaacattgacatctgatccactgctttaggagtgacacaaatgaagttaactcaggctattttctttataatcattgtgctattgttttctttttcttttcaattatactgcttaatataggattttgtggcaccataggagttgag

SEQ ID NO: 9 - DNA, 804 bp, Artificial Sequence
  Enhancer Long
tcgccaccacttggcttccggcacgtggggcagatgtttccattcccacggcggcagcggaagagggagggccgggcgcgccgcggctgcttgcagtctccgcaagcggctacatcacagagctcagcgtgcggtgtcacaggccccgcggtcccgcccaacagatgcaccgagatgcgcgtgcgcagaaagcgtcccgggggtgaggctccctccctcgctctccctctactcccgccccactctcccccactttcccccctccacccaccgcggccgtcggggctcgctcgctcagtacctggaggcgagttcctgacgcgactgcgactcaatcctcgcctggtgaagaatattttacctatgactcactgaaaataaagacggctgagtgaccgtgtttgttcatgtaaacattgaacaaatatttatcggcttctgcgatgtgtcctactcttttagtggaggaagacacattttatttatgtatttaatttttcttttgaattttacatgcgagttatacttaataaaactcacttcaaaatataccttcaacagaaaatccagcaacagtttctattatgttagttaaaacagccagtcttttcctttacttttaaaaattattcataaatgtaattagtgaatgataataaacattgacatctgatccactgctttaggagtgacacaaatgaagttaactcaggctattttctttataatcattgtgctattgttttctttttcttttcaattatactgcttaatataggattttgtggcaccataggagttgag

SEQ ID NO: 10 - DNA, 4429 bp, Artificial Sequence
  Full 5' FVIII promoter sequence
tcgccaccacttggcttccggcacgtggggcagatgtttccattcccacggcggcagcggaagagggagggccgggcgcgccgcggctgcttgcagtctccgcaagcggctacatcacagagctcagcgtgcggtgtcacaggccccgcggtcccgcccaacagatgcaccgagatgcgcgtgcgcagaaagcgtcccgggggtgaggctccctccctcgctctccctctactcccgccccactctcccccactttcccccctccacccaccgcggccgtcggggctcgctcgctcagtacctggaggcgagttcctgacgcgactgcgactcaatcctcgcctggtgaagaatattttacctatgactcactgaaaataaagacggctgagtgaccgtgtttgttcatgtaaacattgaacaaatatttatcggcttctgcgatgtgtcctactcttttagtggaggaagacacattttatttatgtatttaatttttcttttgaattttacatgcgagttatacttaataaaactcacttcaaaatataccttcaacagaaaatccagcaacagtttctattatgttagttaaaacagccagtcttttcctttacttttaaaaattattcataaatgtaattagtgaatgataataaacattgacatctgatccactgctttaggagtgacacaaatgaagttaactcaggctattttctttataatcattgtgctattgttttctttttcttttcaattatactgcttaatataggattttgtggcaccataggagttgagtaaaaataaaaggaataaaaatataccttatctggccgggcgcggtggctcacgcctgtaatttcagcagtttcggaggccgaggcgggcggatcacgcggtcaggagatcgaggccatcctggctaacatggtgaaaccccgtctctactaaaaatacaaaaaattagccgggcatggtggcggccgcctgtagtcccagctactcgggaggctgaggcaggagaatggcgtgaacccgggaggcggagcttgcagtgagccgagatcgcgacactgcactccagcctgggcgacagagtgagactgcgtctccaaaaaaaaaagaaaaaatacgttatctatgaagatttccaatttgatttctatttatcacaaatggccacagtactcctttgtactttaccacataccatattgtattcagtaattatttgtgaatatgtaattgataatattgtaggttttagagaatccttgaaaacatgaaaatttggtaatggggtctattttgattatttatttatttatttatttattttatttttgagacagagtctcgctcttgttgcccaggctggagtgcagtggcgcgatctcggctcactgcaagctccacctcccgggttcaagcgattctcctgcctcagcctcccaagtagctgggactacaggcacgtgccaccatgcccggctaattttttgtatttttagtagaggaggagtttcatcttgttagctaggatggtctagatctcctgacctcgtgatctgcccgcctcagcctcccaaagtgctgggattacaggtgtgagccaccgtgcccggccatattttgatttaaaatttagcaataatagataaaattttcaatcaactaagcccttgggccagggaatgctattccttaaaaagtgcttctatcaatatagcctctgactcattactttgttaatttttaaattgtatttcattcctgattaacattcccacccagattattaattatacaatctgttaactgtagaacctcaaacatgttggattgtactgtatttgtctggaagacacatttttaaaacattgtaatcgctataagagaagcactgggaaagaaaggagcttctatgcctgcagtgcctgaggagccctttaacagtgtgccccgcccctaagctactcatgcagtcatccccatcccagttagtcaactttattccaaaaaacttggtgttccaaatttttccttctcaaagcccacagatccaaaattcatcagcagttcccacaaacgttaccctcacaatgaatccagccatttttcaccctctccagtggtaccatcatagcccaagccgccaccatttctcacccccggttaacaggccaccctccttctacccttatcctgctagagtttgttttatctacagtgatcagaaagatcagcctaaaagataattctgatcaccaccctcctctactcacaacccggccgtgtctccccattgccctcagtgtagaagtcaatgtccctttgctgaaatgcaaccttagtgaaactttccatgactaacctcctttaaaattgcaacctggtccacccttactcccccttaccccacttctcttttttgcacagcacttattttaccttctaacatactgtataatgtactcatgtattgtaattattgcttatcatccctctttcagttgcttatatttttcatcaatgtgtacccagtgcctaggacaatatctgtctaggacaaatgggtagttatgtggctgtaggcaagccatttaacctctctgtacctcagttactttatctgtatccactttgcggtgttgtcatgaggattaaatcagatagcctatgtgtagcacctggcagtgaatttatcaccctgtactgtaactgtctacttttctgtctcctccattggactgtcattcccagggggttgggaactgggatttcttcatttctgaggcatagaagtatagcatagtggttaggagcatgacttctggagccagagtacatgggtttgaatgctaccactcacaagctgtgtggccatggagaagttgcctaacctctccgtgcttcagtttcatcacccataaaatgaaggtaagaatagtacctgtatttaaaagcacctagaacagttcctggcatatagtgtcagctgtcatctctgcatccttgtacctgtcagagaggagtgtttatcaaaggggcttcttgctgcctgtttccaaaccagtcgacaatataccaattgctccctaacacattcttgtttgtgcagaactgagctcaatgataacatttttatagcaaccctgatcaagtttcttctcataatctcttacactttgaggcccctgcaggggccctcactctccctaataaacattaacctgagtagggtgtttgagctcaccatggctacattctgatgtaaagagatatatcctatacctgggccaaatgtaaacagcctggaaaagtgttaggttaaaaacaaaacaaaataaataaatgaataaatgccaggtggttatgagtgctattgagaaaaatgaagccaagagggatatcagtgatgcaggtgggggtaaagagcttacaacataaatgtggtgttccatatttaaacctcattcaacagggaagattggagctgaaatgtgaaggagttgtgggagtggaactacgtggaaatctgggggaaaggtgttttgggtaaaagaaatagcaagtgttgaggtccaggggcatgagtgtgcttgatattttagggaagagtaaggagaccagtataaccagagtgagatgagactacagaggtcaggagaaagggcatgcagaccatgtgggatgctctaggacctaggccatggtaaagatgtagggttttaccctgatggaggtcagaagccattggaggattctgagaagaggagtgacaggactcgctttatagttttaaattataactataaattatagtttttaaaacaatagttgcctaacctcatgttatatgtaaaactacagttttaaaaactataaattcctcatactggcagcagtgtgaggggcaagggcaaaagcagagagactaacaggttgctggttactcttgctagtgcaagtgaattctagaatcttcgacaacatccagaacttctcttgctgctgccactcaggaagagggttggagtaggctaggaataggagcacaaattaaagctcctgttcactttgacttctccatccctctcctcctttccttaaaggttctgattaaagcagacttatgcccctactgctctcagaagtgaatgggttaagtttagcagcctcccttttgctacttcagttcttcctgtggctgcttcccactgataaaaaggaagcaatcctatcggttactgcttagtgctgagcacatccagtgggtaaagttccttaaaatgctctgcaaagaaattgggacttttcattaaatcagaaattttacttttttcccctcctgggagctaaagatattttagagaagaattaaccttttgcttctccagttgaacatttgtagcaataagtc

SEQ ID NO: 11 - DNA, 4374 bp, Artificial Sequence
  BDD FVIII
atgcaaatagagctctccacctgcttctttctgtgccttttgcgattctgctttagtgccaccagaagatactacctgggtgcagtggaactgtcatgggactatatgcaaagtgatctcggtgagctgcctgtggacgcaagatttcctcctagagtgccaaaatcttttccattcaacacctcagtcgtgtacaaaaagactctgtttgtagaattcacggatcaccttttcaacatcgctaagccaaggccaccctggatgggtctgctaggtcctaccatccaggctgaggtttatgatacagtggtcattacacttaagaacatggcttcccatcctgtcagtcttcatgctgttggtgtatcctactggaaagcttctgagggagctgaatatgatgatcagaccagtcaaagggagaaagaagatgataaagtcttccctggtggaagccatacatatgtctggcaggtcctgaaagagaatggtccaatggcctctgacccactgtgccttacctactcatatctttctcatgtggacctggtaaaagacttgaattcaggcctcattggagccctactagtatgtagagaagggagtctggccaaggaaaagacacagaccttgcacaaatttatactactttttgctgtatttgatgaagggaaaagttggcactcagaaacaaagaactccttgatgcaggatagggatgctgcatctgctcgggcctggcctaaaatgcacacagtcaatggttatgtaaacaggtctctgccaggtctgattggatgccacaggaaatcagtctattggcatgtgattggaatgggcaccactcctgaagtgcactcaatattcctcgaaggtcacacatttcttgtgaggaaccatcgccaggcgtccttggaaatctcgccaataactttccttactgctcaaacactcttgatggaccttggacagtttctactgttttgtcatatctcttcccaccaacatgatggcatggaagcttatgtcaaagtagacagctgtccagaggaaccccaactacgaatgaaaaataatgaagaagcggaagactatgatgatgatcttactgattctgaaatggatgtggtcaggtttgatgatgacaactctccttcctttatccaaattcgctcagttgccaagaagcatcctaaaacttgggtacattacattgctgctgaagaggaggactgggactatgctcccttagtcctcgcccccgatgacagaagttataaaagtcaatatttgaacaatggccctcagcggattggtaggaagtacaaaaaagtccgatttatggcatacacagatgaaacctttaagactcgtgaagctattcagcatgaatcaggaatcttgggacctttactttatggggaagttggagacacactgttgattatatttaagaatcaagcaagcagaccatataacatctaccctcacggaatcactgatgtccgtcctttgtattcaaggagattaccaaaaggtgtaaaacatttgaaggattttccaattctgccaggagaaatattcaaatataaatggacagtgactgtagaagatgggccaactaaatcagatcctcggtgcctgacccgctattactctagtttcgttaatatggagagagatctagcttcaggactcattggccctctcctcatctgctacaaagaatctgtagatcaaagaggaaaccagataatgtcagacaagaggaatgtcatcctgttttctgtatttgatgagaaccgaagctggtacctcacagagaatatacaacgctttctccccaatccagctggagtgcagcttgaggatccagagttccaagcctccaacatcatgcacagcatcaatggctatgtttttgatagtttgcagttgtcagtttgtttgcatgaggtggcatactggtacattctaagcattggagcacagactgacttcctttctgtcttcttctctggatataccttcaaacacaaaatggtctatgaagacacactcaccctattcccattctcaggagaaactgtcttcatgtcgatggaaaacccaggtctatggattctggggtgccacaactcagactttcggaacagaggcatgaccgccttactgaaggtttctagttgtgacaagaacactggtgattattacgaggacagttatgaagatatttcagcatacttgctgagtaaaaacaatgccattgaaccaagaagcttctcccaaaacccaccagtcttgaaacgccatcaacgggaaataactcgtactactcttcagtcagatcaagaggaaattgactatgatgataccatatcagttgaaatgaagaaggaagattttgacatttatgatgaggatgaaaatcagagcccccgcagctttcaaaagaaaacacgacactattttattgctgcagtggagaggctctgggattatgggatgagtagctccccacatgttctaagaaacagggctcagagtggcagtgtccctcagttcaagaaagttgttttccaggaatttactgatggctcctttactcagcccttataccgtggagaactaaatgaacatttgggactcctggggccatatataagagcagaagttgaagataatatcatggtaactttcagaaatcaggcctctcgtccctattccttctattctagccttatttcttatgaggaagatcagaggcaaggagcagaacctagaaaaaactttgtcaagcctaatgaaaccaaaacttacttttggaaagtgcaacatcatatggcacccactaaagatgagtttgactgcaaagcctgggcttatttctctgatgttgacctggaaaaagatgtgcactcaggcctgattggaccccttctggtctgccacactaacacactgaaccctgctcatgggagacaagtgacagtacaggaatttgctctgtttttcaccatctttgatgagaccaaaagctggtacttcactgaaaatatggaaagaaactgcagggctccctgcaatatccagatggaagatcccacttttaaagagaattatcgcttccatgcaatcaatggctacataatggatacactacctggcttagtaatggctcaggatcaaaggattcgatggtatctgctcagcatgggcagcaatgaaaacatccattctattcatttcagtggacatgtgttcaccgtacgaaaaaaagaggagtataaaatggcactgtacaatctctatccaggtgtttttgagacagtggaaatgttaccatccaaagctggaatttggcgggtggaatgccttattggcgagcatctacatgctgggatgagcacactttttctggtgtacagcaataagtgtcagactcccctgggaatggcttctggacacattagagattttcagattacagcttcaggacaatatggacagtgggccccaaagctggccagacttcattattccggatcaatcaatgcctggagcaccaaggagcccttttcttggatcaaggtggatctgttggcaccaatgattattcacggcatcaagacccagggtgcccgtcagaagttctccagcctctacatctctcagtttatcatcatgtatagtcttgatgggaagaagtggcagacttatcgaggaaattccactggaaccttaatggtcttctttggcaatgtggattcatctgggataaaacacaatatttttaaccctccaattattgctcgatacatccgtttgcacccaactcattatagcattcgcagcactcttcgcatggagttgatgggctgtgatttaaatagttgcagcatgccattgggaatggagagtaaagcaatatcagatgcacagattactgcttcatcctactttaccaatatgtttgccacctggtctccttcaaaagctcgacttcacctccaagggaggagtaatgcctggagacctcaggtgaataatccaaaagagtggctgcaagtggacttccagaagacaatgaaagtcacaggagtaactactcagggagtaaaatctctgcttaccagcatgtatgtgaaggagttcctcatctccagcagtcaagatggccatcagtggactctcttttttcagaatggcaaagtaaaggtttttcagggaaatcaagactccttcacacctgtggtgaactctctagacccaccgttactgactcgctaccttcgaattcacccccagagttgggtgcaccagattgccctgaggatggaggttctgggctgcgaggcacaggacctctactga

SEQ ID NO: 12 - DNA, 442 bp, Artificial Sequence
  LV.pF8.8
aatcttcgacaacatccagaacttctcttgctgctgccactcaggaagagggttggagtaggctaggaataggagcacaaattaaagctcctgttcactttgacttctccatccctctcctcctttccttaaaggttctgattaaagcagacttatgcccctactgctctcagaagtgaatgggttaagtttagcagcctcccttttgctacttcagttcttcctgtggctgcttcccactgataaaaaggaagcaatcctatcggttactgcttagtgctgagcacatccagtgggtaaagttccttaaaatgctctgcaaagaaattgggacttttcattaaatcagaaattttacttttttcccctcctgggagctaaagatattttagagaagaattaaccttttgcttctccagttgaacatttgtagcaataagtc

SEQ ID NO: 13 - DNA, 4785 bp, Artificial Sequence
  FVIII-N6
atgcaaagtgatctcggtgagctgcctgtggacgcaagatttcctcctagagtgccaaaatcttttccattcaacacctcagtcgtgtacaaaaagactctgtttgtagaattcacggatcaccttttcaacatcgctaagccaaggccaccctggatgggtctgctaggtcctaccatccaggctgaggtttatgatacagtggtcattacacttaagaacatggcttcccatcctgtcagtcttcatgctgttggtgtatcctactggaaagcttctgagggagctgaatatgatgatcagaccagtcaaagggagaaagaagatgataaagtcttccctggtggaagccatacatatgtctggcaggtcctgaaagagaatggtccaatggcctctgacccactgtgccttacctactcatatctttctcatgtggacctggtaaaagacttgaattcaggcctcattggagccctactagtatgtagagaagggagtctggccaaggaaaagacacagaccttgcacaaatttatactactttttgctgtatttgatgaagggaaaagttggcactcagaaacaaagaactccttgatgcaggatagggatgctgcatctgctcgggcctggcctaaaatgcacacagtcaatggttatgtaaacaggtctctgccaggtctgattggatgccacaggaaatcagtctattggcatgtgattggaatgggcaccactcctgaagtgcactcaatattcctcgaaggtcacacatttcttgtgaggaaccatcgccaggcgtccttggaaatctcgccaataactttccttactgctcaaacactcttgatggaccttggacagtttctactgtcttgtcatatctcttcccaccaacatgatggcatggaagcttatgtcaaagtagacagctgtccagaggaaccccaactacgaatgaaaaataatgaagaagcggaagactatgatgatgatcttactgattctgaaatggatgtggtcaggtttgatgatgacaactctccttcctttatccaaattcgctcagttgccaagaagcatcctaaaacttgggtacattacattgctgctgaagaggaggactgggactatgctcccttagtcctcgcccccgatgacagaagttataaaagtcaatatttgaacaatggccctcagcggattggtaggaagtacaaaaaagtccgatttatggcatacacagatgaaacctttaagactcgtgaagctattcagcatgaatcaggaatcttgggacctttactttatggggaagttggagacacactgttgattatatttaagaatcaagcaagcagaccatataacatctaccctcacggaatcactgatgtccgtcctttgtattcaaggagattaccaaaaggtgtaaaacatttgaaggattttccaattctgccaggagaaatattcaaatataaatggacagtgactgtagaagatgggccaactaaatcagatcctcggtgcctgacccgctattactctagtttcgttaatatggagagagatctagcttcaggactcattggccctctcctcatctgctacaaagaatctgtagatcaaagaggaaaccagataatgtcagacaagaggaatgtcatcctgttttctgtatttgatgagaaccgaagctggtacctcacagagaatatacaacgctttctccccaatccagctggagtgcagcttgaggatccagagttccaagcctccaacatcatgcacagcatcaatggctatgtttttgatagtttgcagttgtcagtttgtttgcatgaggtggcatactggtacattctaagcattggagcacagactgacttcctttctgtcttcttctctggatataccttcaaacacaaaatggtctatgaagacacactcaccctattcccattctcaggagaaactgtcttcatgtcgatggaaaacccaggtctatggattctggggtgccacaactcagactttcggaacagaggcatgaccgccttactgaaggtttctagttgtgacaagaacactggtgattattacgaggacagttatgaagatatttcagcatacttgctgagtaaaaacaatgccattgaaccaagaagcttctcccagaattcaagacaccctagcactaggcaaaagcaatttaatgccaccacaattccagaaaatgacatagagaagactgacccttggtttgcacacagaacacctatgcctaaaatacaaaatgtctcctctagtgatttgttgatgctcttgcgacagagtcctactccacatgggctatccttatctgatctccaagaagccaaatatgagactttttctgatgatccatcacctggagcaatagacagtaataacagcctgtctgaaatgacacacttcaggccacagctccatcacagtggggacatggtatttacccctgagtcaggcctccaattaagattaaatgagaaactggggacaactgcagcaacagagttgaagaaacttgatttcaaagtttctagtacatcaaataatctgatttcaacaattccatcagacaatttggcagcaggtactgataatacaagttccttaggacccccaagtatgccagttcattatgatagtcaattagataccactctatttggcaaaaagtcatctccccttactgagtctggtggacctctgagcttgagtgaagaaaataatgattcaaagttgttagaatcaggtttaatgaatagccaagaaagttcatggggaaaaaatgtatcgacgcgtagctttcaaaagaaaacacgacactattttattgctgcagtggagaggctctgggattatgggatgagtagctccccacatgttctaagaaacagggctcagagtggcagtgtccctcagttcaagaaagttgttttccaggaatttactgatggctcctttactcagcccttataccgtggagaactaaatgaacatttgggactcctggggccatatataagagcagaagttgaagataatatcatggtaactttcagaaatcaggcctctcgtccctattccttctattctagccttatttcttatgaggaagatcagaggcaaggagcagaacctagaaaaaactttgtcaagcctaatgaaaccaaaacttacttttggaaagtgcaacatcatatggcacccactaaagatgagtttgactgcaaagcctgggcttatttctctgatgttgacctggaaaaagatgtgcactcaggcctgattggaccccttctggtctgccacactaacacactgaaccctgctcatgggagacaagtgacagtacaggaatttgctctgtttttcaccatctttgatgagaccaaaagctggtacttcactgaaaatatggaaagaaactgcagggctccctgcaatatccagatggaagatcccacttttaaagagaattatcgcttccatgcaatcaatggctacataatggatacactacctggcttagtaatggctcaggatcaaaggattcgatggtatctgctcagcatgggcagcaatgaaaacatccattctattcatttcagtggacatgtgttcactgtacgaaaaaaagaggagtataaaatggcactgtacaatctctatccaggtgtttttgagacagtggaaatgttaccatccaaagctggaatttggcgggtggaatgccttattggcgagcatctacatgctgggatgagcacactttttctggtgtacagcaataagtgtcagactcccctgggaatggcttctggacacattagagattttcagattacagcttcaggacaatatggacagtgggccccaaagctggccagacttcattattccggatcaatcaatgcctggagcaccaaggagcccttttcttggatcaaggtggatctgttggcaccaatgattattcacggcatcaagacccagggtgcccgtcagaagttctccagcctctacatctctcagtttatcatcatgtatagtcttgatgggaagaagtggcagacttatcgaggaaattccactggaaccttaatggtcttctttggcaatgtggattcatctgggataaaacacaatatttttaaccctccaattattgctcgatacatccgtttgcacccaactcattatagcattcgcagcactcttcgcatggagttgatgggctgtgatttaaatagttgcagcatgccattgggaatggagagtaaagcaatatcagatgcacagattactgcttcatcctactttaccaatatgtttgccacctggtctccttcaaaagctcgacttcacctccaagggaggagtaatgcctggagacctcaggtgaataatccaaaagagtggctgcaagtggacttccagaagacaatgaaagtcacaggagtaactactcagggagtaaaatctctgcttaccagcatgtatgtgaaggagttcctcatctccagcagtcaagatggccatcagtggactctcttttttcagaatggcaaagtaaaggtttttcagggaaatcaagactccttcacacctgtggtgaactctctagacccaccgttactgactcgctaccttcgaattcacccccagagttgggtgcaccagattgccctgaggatggaggttctgggctgcgaggcacaggacctctactga

SEQ ID NO: 14 - DNA, 4374 bp, Artificial Sequence
  FVIII-RH
atgcaaatagagctctccacctgcttctttctgtgccttttgcgattctgctttagtgccaccagaagatactacctgggtgcagtggaactgtcatgggactatatgcaaagtgatctcggtgagctgcctgtggacgcaagatttcctcctagagtgccaaaatcttttccattcaacacctcagtcgtgtacaaaaagactctgtttgtagaattcacggatcaccttttcaacatcgctaagccaaggccaccctggatgggtctgctaggtcctaccatccaggctgaggtttatgatacagtggtcattacacttaagaacatggcttcccatcctgtcagtcttcatgctgttggtgtatcctactggaaagcttctgagggagctgaatatgatgatcagaccagtcaaagggagaaagaagatgataaagtcttccctggtggaagccatacatatgtctggcaggtcctgaaagagaatggtccaatggcctctgacccactgtgccttacctactcatatctttctcatgtggacctggtaaaagacttgaattcaggcctcattggagccctactagtatgtagagaagggagtctggccaaggaaaagacacagaccttgcacaaatttatactactttttgctgtatttgatgaagggaaaagttggcactcagaaacaaagaactccttgatgcaggatagggatgctgcatctgctcgggcctggcctaaaatgcacacagtcaatggttatgtaaacaggtctctgccaggtctgattggatgccacaggaaatcagtctattggcatgtgattggaatgggcaccactcctgaagtgcactcaatattcctcgaaggtcacacatttcttgtgaggaaccatcgccaggcgtccttggaaatctcgccaataactttccttactgctcaaacactcttgatggaccttggacagtttctactgttttgtcatatctcttcccaccaacatgatggcatggaagcttatgtcaaagtagacagctgtccagaggaaccccaactacgaatgaaaaataatgaagaagcggaagactatgatgatgatcttactgattctgaaatggatgtggtcaggtttgatgatgacaactctccttcctttatccaaattcgctcagttgccaagaagcatcctaaaacttgggtacattacattgctgctgaagaggaggactgggactatgctcccttagtcctcgcccccgatgacagaagttataaaagtcaatatttgaacaatggccctcagcggattggtaggaagtacaaaaaagtccgatttatggcatacacagatgaaacctttaagactcgtgaagctattcagcatgaatcaggaatcttgggacctttactttatggggaagttggagacacactgttgattatatttaagaatcaagcaagcagaccatataacatctaccctcacggaatcactgatgtccgtcctttgtattcaaggagattaccaaaaggtgtaaaacatttgaaggattttccaattctgccaggagaaatattcaaatataaatggacagtgactgtagaagatgggccaactaaatcagatcctcggtgcctgacccgctattactctagtttcgttaatatggagagagatctagcttcaggactcattggccctctcctcatctgctacaaagaatctgtagatcaaagaggaaaccagataatgtcagacaagaggaatgtcatcctgttttctgtatttgatgagaaccgaagctggtacctcacagagaatatacaacgctttctccccaatccagctggagtgcagcttgaggatccagagttccaagcctccaacatcatgcacagcatcaatggctatgtttttgatagtttgcagttgtcagtttgtttgcatgaggtggcatactggtacattctaagcattggagcacagactgacttcctttctgtcttcttctctggatataccttcaaacacaaaatggtctatgaagacacactcaccctattcccattctcaggagaaactgtcttcatgtcgatggaaaacccaggtctatggattctggggtgccacaactcagactttcggaacagaggcatgaccgccttactgaaggtttctagttgtgacaagaacactggtgattattacgaggacagttatgaagatatttcagcatacttgctgagtaaaaacaatgccattgaaccaagaagcttctcccaaaacccaccagtcttgaaacaccatcaacgggaaataactcgtactactcttcagtcagatcaagaggaaattgactatgatgataccatatcagttgaaatgaagaaggaagattttgacatttatgatgaggatgaaaatcagagcccccgcagctttcaaaagaaaacacgacactattttattgctgcagtggagaggctctgggattatgggatgagtagctccccacatgttctaagaaacagggctcagagtggcagtgtccctcagttcaagaaagttgttttccaggaatttactgatggctcctttactcagcccttataccgtggagaactaaatgaacatttgggactcctggggccatatataagagcagaagttgaagataatatcatggtaactttcagaaatcaggcctctcgtccctattccttctattctagccttatttcttatgaggaagatcagaggcaaggagcagaacctagaaaaaactttgtcaagcctaatgaaaccaaaacttacttttggaaagtgcaacatcatatggcacccactaaagatgagtttgactgcaaagcctgggcttatttctctgatgttgacctggaaaaagatgtgcactcaggcctgattggaccccttctggtctgccacactaacacactgaaccctgctcatgggagacaagtgacagtacaggaatttgctctgtttttcaccatctttgatgagaccaaaagctggtacttcactgaaaatatggaaagaaactgcagggctccctgcaatatccagatggaagatcccacttttaaagagaattatcgcttccatgcaatcaatggctacataatggatacactacctggcttagtaatggctcaggatcaaaggattcgatggtatctgctcagcatgggcagcaatgaaaacatccattctattcatttcagtggacatgtgttcaccgtacgaaaaaaagaggagtataaaatggcactgtacaatctctatccaggtgtttttgagacagtggaaatgttaccatccaaagctggaatttggcgggtggaatgccttattggcgagcatctacatgctgggatgagcacactttttctggtgtacagcaataagtgtcagactcccctgggaatggcttctggacacattagagattttcagattacagcttcaggacaatatggacagtgggccccaaagctggccagacttcattattccggatcaatcaatgcctggagcaccaaggagcccttttcttggatcaaggtggatctgttggcaccaatgattattcacggcatcaagacccagggtgcccgtcagaagttctccagcctctacatctctcagtttatcatcatgtatagtcttgatgggaagaagtggcagacttatcgaggaaattccactggaaccttaatggtcttctttggcaatgtggattcatctgggataaaacacaatatttttaaccctccaattattgctcgatacatccgtttgcacccaactcattatagcattcgcagcactcttcgcatggagttgatgggctgtgatttaaatagttgcagcatgccattgggaatggagagtaaagcaatatcagatgcacagattactgcttcatcctactttaccaatatgtttgccacctggtctccttcaaaagctcgacttcacctccaagggaggagtaatgcctggagacctcaggtgaataatccaaaagagtggctgcaagtggacttccagaagacaatgaaagtcacaggagtaactactcagggagtaaaatctctgcttaccagcatgtatgtgaaggagttcctcatctccagcagtcaagatggccatcagtggactctcttttttcagaatggcaaagtaaaggtttttcagggaaatcaagactccttcacacctgtggtgaactctctagacccaccgttactgactcgctaccttcgaattcacccccagagttgggtgcaccagattgccctgaggatggaggttctgggctgcgaggcacaggacctctactga

SEQ ID NO: 15 - DNA, 4377 bp, Artificial Sequence
  CodonOptimized (CO) FVIII
atgcagatcgagctgtccacctgcttttttctgtgcctgctgcggttctgcttcagcgccacccggcggtactacctgggcgccgtggagctgtcctgggactacatgcagagcgacctgggcgagctgcccgtggacgcccggttcccccccagagtgcccaagagcttccccttcaacaccagcgtggtgtacaagaaaaccctgttcgtggagttcaccgaccacctgttcaatatcgccaagcccaggcccccctggatgggcctgctgggccccaccatccaggccgaggtgtacgacaccgtggtgatcaccctgaagaacatggccagccaccccgtgagcctgcacgccgtgggcgtgagctactggaaggccagcgagggcgccgagtacgacgaccagaccagccagcgggagaaagaagatgacaaggtgttccctggcggcagccacacctacgtgtggcaggtgctgaaagaaaacggccccatggcctccgaccccctgtgcctgacctacagctacctgagccacgtggacctggtgaaggacctgaacagcggcctgatcggcgctctgctcgtctgccgggagggcagcctggccaaagagaaaacccagaccctgcacaagttcatcctgctgttcgccgtgttcgacgagggcaagagctggcacagcgagacaaagaacagcctgatgcaggaccgggacgccgcctctgccagagcctggcccaagatgcacaccgtgaacggctacgtgaacagaagcctgcccggcctgattggctgccaccggaagagcgtgtactggcacgtgatcggcatgggcaccacacccgaggtgcacagcatctttctggaagggcacacctttctggtccggaaccaccggcaggccagcctggaaatcagccctatcaccttcctgaccgcccagacactgctgatggacctgggccagttcctgctgttttgccacatcagctctcaccagcacgacggcatggaagcctacgtgaaggtggactcttgccccgaggaaccccagctgcggatgaagaacaacgaggaagccgaggactacgacgacgacctgaccgacagcgagatggacgtggtgcggttcgacgacgacaacagccccagcttcatccagatcagaagcgtggccaagaagcaccccaagacctgggtgcactatatcgccgccgaggaagaggactgggactacgcccccctggtgctggcccccgacgacagaagctacaagagccagtacctgaacaatggcccccagcggatcggccggaagtacaagaaagtgcggttcatggcctacaccgacgagacattcaagacccgggaggccatccagcacgagagcggcatcctgggccccctgctgtacggcgaagtgggcgacacactgctgatcatcttcaagaaccaggctagccggccctacaacatctacccccacggcatcaccgacgtgcggcccctgtacagcaggcggctgcccaagggcgtgaagcacctgaaggacttccccatcctgcccggcgagatcttcaagtacaagtggaccgtgaccgtggaggacggccccaccaagagcgaccccagatgcctgacccggtactacagcagcttcgtgaacatggaacgggacctggcctccgggctgatcggacctctgctgatctgctacaaagaaagcgtggaccagcggggcaaccagatcatgagcgacaagcggaacgtgatcctgttcagcgtgttcgatgagaaccggtcctggtatctgaccgagaacatccagcggtttctgcccaaccctgccggcgtgcagctggaagatcccgagttccaggccagcaacatcatgcactccatcaatggctacgtgttcgactctctgcagctctccgtgtgtctgcacgaggtggcctactggtacatcctgagcatcggcgcccagaccgacttcctgagcgtgttcttcagcggctacaccttcaagcacaagatggtgtacgaggacaccctgaccctgttccctttcagcggcgagacagtgttcatgagcatggaaaaccccggcctgtggattctgggctgccacaacagcgacttccggaaccggggcatgaccgccctgctgaaggtgtccagctgcgacaagaacaccggcgactactacgaggacagctacgaggatatcagcgcctacctgctgtccaagaacaacgccatcgaaccccggagcttcagccagaacccccccgtgctgacgcgtcaccagcgggagatcacccggacaaccctgcagtccgaccaggaagagatcgattacgacgacaccatcagcgtggagatgaagaaagaggatttcgatatctacgacgaggacgagaaccagagccccagaagcttccagaagaaaacccggcactacttcattgccgccgtggagaggctgtgggactacggcatgagttctagcccccacgtgctgcggaaccgggcccagagcggcagcgtgccccagttcaagaaagtggtgttccaggaattcacagacggcagcttcacccagcctctgtatagaggcgagctgaacgagcacctggggctgctggggccctacatcagggccgaagtggaggacaacatcatggtgaccttccggaatcaggccagcagaccctactccttctacagcagcctgatcagctacgaagaggaccagcggcagggcgccgaaccccggaagaacttcgtgaagcccaacgaaaccaagacctacttctggaaagtgcagcaccacatggcccccaccaaggacgagttcgactgcaaggcctgggcctacttcagcgacgtggatctggaaaaggacgtgcactctggactgattggcccactcctggtctgccacactaacaccctcaaccccgcccacggccgccaggtgaccgtgcaggaattcgccctgttcttcaccatcttcgacgagacaaagtcctggtacttcaccgagaatatggaacggaactgcagagccccctgcaacatccagatggaagatcctaccttcaaagagaactaccggttccacgccatcaacggctacatcatggacaccctgcctggcctggtgatggcccaggaccagagaatccggtggtatctgctgtccatgggcagcaacgagaatatccacagcatccacttcagcggccacgtgttcaccgtgcggaagaaagaagagtacaagatggccctgtacaacctgtaccccggcgtgttcgagacagtggagatgctgcccagcaaggccggcatctggcgggtggagtgtctgatcggcgagcacctgcacgctggcatgagcaccctgtttctggtgtacagcaacaagtgccagaccccactgggcatggcctctggccacatccgggacttccagatcaccgcctccggccagtacggccagtgggcccccaagctggccagactgcactacagcggcagcatcaacgcctggtccaccaaagagcccttcagctggatcaaggtggacctgctggcccctatgatcatccacggcattaagacccagggcgccaggcagaagttcagcagcctgtacatcagccagttcatcatcatgtacagcctggacggcaagaagtggcagacctaccggggcaacagcaccggcaccctgatggtgttcttcggcaatgtggacagcagcggcatcaagcacaacatcttcaacccccccatcattgcccggtacatccggctgcaccccacccactacagcattagatccacactgagaatggaactgatgggctgcgacctgaactcctgcagcatgcctctgggcatggaaagcaaggccatcagcgacgcccagatcacagccagcagctacttcaccaacatgttcgccacctggtccccctccaaggccaggctgcacctgcagggccggtccaacgcctggcggcctcaggtcaacaaccccaaagaatggctgcaggtggactttcagaaaaccatgaaggtgaccggcgtgaccacccagggcgtgaaaagcctgctgaccagcatgtacgtgaaagagtttctgatcagcagctctcaggatggccaccagtggaccctgttctttcagaacggcaaggtgaaagtgttccagggcaaccaggactccttcacccccgtggtgaactccctggacccccccctgctgacccgctacctgagaatccacccccagtcttgggtgcaccagatcgccctcaggatggaagtcctgggatgtgaggcccaggatctgtactgatga

SEQ ID NO: 16 - DNA, 4377 bp, Artificial Sequence
  CO FVIII-RH
atgcagatcgagctgtccacctgcttttttctgtgcctgctgcggttctgcttcagcgccacccggcggtactacctgggcgccgtggagctgtcctgggactacatgcagagcgacctgggcgagctgcccgtggacgcccggttcccccccagagtgcccaagagcttccccttcaacaccagcgtggtgtacaagaaaaccctgttcgtggagttcaccgaccacctgttcaatatcgccaagcccaggcccccctggatgggcctgctgggccccaccatccaggccgaggtgtacgacaccgtggtgatcaccctgaagaacatggccagccaccccgtgagcctgcacgccgtgggcgtgagctactggaaggccagcgagggcgccgagtacgacgaccagaccagccagcgggagaaagaagatgacaaggtgttccctggcggcagccacacctacgtgtggcaggtgctgaaagaaaacggccccatggcctccgaccccctgtgcctgacctacagctacctgagccacgtggacctggtgaaggacctgaacagcggcctgatcggcgctctgctcgtctgccgggagggcagcctggccaaagagaaaacccagaccctgcacaagttcatcctgctgttcgccgtgttcgacgagggcaagagctggcacagcgagacaaagaacagcctgatgcaggaccgggacgccgcctctgccagagcctggcccaagatgcacaccgtgaacggctacgtgaacagaagcctgcccggcctgattggctgccaccggaagagcgtgtactggcacgtgatcggcatgggcaccacacccgaggtgcacagcatctttctggaagggcacacctttctggtccggaaccaccggcaggccagcctggaaatcagccctatcaccttcctgaccgcccagacactgctgatggacctgggccagttcctgctgttttgccacatcagctctcaccagcacgacggcatggaagcctacgtgaaggtggactcttgccccgaggaaccccagctgcggatgaagaacaacgaggaagccgaggactacgacgacgacctgaccgacagcgagatggacgtggtgcggttcgacgacgacaacagccccagcttcatccagatcagaagcgtggccaagaagcaccccaagacctgggtgcactatatcgccgccgaggaagaggactgggactacgcccccctggtgctggcccccgacgacagaagctacaagagccagtacctgaacaatggcccccagcggatcggccggaagtacaagaaagtgcggttcatggcctacaccgacgagacattcaagacccgggaggccatccagcacgagagcggcatcctgggccccctgctgtacggcgaagtgggcgacacactgctgatcatcttcaagaaccaggctagccggccctacaacatctacccccacggcatcaccgacgtgcggcccctgtacagcaggcggctgcccaagggcgtgaagcacctgaaggacttccccatcctgcccggcgagatcttcaagtacaagtggaccgtgaccgtggaggacggccccaccaagagcgaccccagatgcctgacccggtactacagcagcttcgtgaacatggaacgggacctggcctccgggctgatcggacctctgctgatctgctacaaagaaagcgtggaccagcggggcaaccagatcatgagcgacaagcggaacgtgatcctgttcagcgtgttcgatgagaaccggtcctggtatctgaccgagaacatccagcggtttctgcccaaccctgccggcgtgcagctggaagatcccgagttccaggccagcaacatcatgcactccatcaatggctacgtgttcgactctctgcagctctccgtgtgtctgcacgaggtggcctactggtacatcctgagcatcggcgcccagaccgacttcctgagcgtgttcttcagcggctacaccttcaagcacaagatggtgtacgaggacaccctgaccctgttccctttcagcggcgagacagtgttcatgagcatggaaaaccccggcctgtggattctgggctgccacaacagcgacttccggaaccggggcatgaccgccctgctgaaggtgtccagctgcgacaagaacaccggcgactactacgaggacagctacgaggatatcagcgcctacctgctgtccaagaacaacgccatcgaaccccggagcttcagccagaacccccccgtgctgacgcatcaccagcgggagatcacccggacaaccctgcagtccgaccaggaagagatcgattacgacgacaccatcagcgtggagatgaagaaagaggatttcgatatctacgacgaggacgagaaccagagccccagaagcttccagaagaaaacccggcactacttcattgccgccgtggagaggctgtgggactacggcatgagttctagcccccacgtgctgcggaaccgggcccagagcggcagcgtgccccagttcaagaaagtggtgttccaggaattcacagacggcagcttcacccagcctctgtatagaggcgagctgaacgagcacctggggctgctggggccctacatcagggccgaagtggaggacaacatcatggtgaccttccggaatcaggccagcagaccctactccttctacagcagcctgatcagctacgaagaggaccagcggcagggcgccgaaccccggaagaacttcgtgaagcccaacgaaaccaagacctacttctggaaagtgcagcaccacatggcccccaccaaggacgagttcgactgcaaggcctgggcctacttcagcgacgtggatctggaaaaggacgtgcactctggactgattggcccactcctggtctgccacactaacaccctcaaccccgcccacggccgccaggtgaccgtgcaggaattcgccctgttcttcaccatcttcgacgagacaaagtcctggtacttcaccgagaatatggaacggaactgcagagccccctgcaacatccagatggaagatcctaccttcaaagagaactaccggttccacgccatcaacggctacatcatggacaccctgcctggcctggtgatggcccaggaccagagaatccggtggtatctgctgtccatgggcagcaacgagaatatccacagcatccacttcagcggccacgtgttcaccgtgcggaagaaagaagagtacaagatggccctgtacaacctgtaccccggcgtgttcgagacagtggagatgctgcccagcaaggccggcatctggcgggtggagtgtctgatcggcgagcacctgcacgctggcatgagcaccctgtttctggtgtacagcaacaagtgccagaccccactgggcatggcctctggccacatccgggacttccagatcaccgcctccggccagtacggccagtgggcccccaagctggccagactgcactacagcggcagcatcaacgcctggtccaccaaagagcccttcagctggatcaaggtggacctgctggcccctatgatcatccacggcattaagacccagggcgccaggcagaagttcagcagcctgtacatcagccagttcatcatcatgtacagcctggacggcaagaagtggcagacctaccggggcaacagcaccggcaccctgatggtgttcttcggcaatgtggacagcagcggcatcaagcacaacatcttcaacccccccatcattgcccggtacatccggctgcaccccacccactacagcattagatccacactgagaatggaactgatgggctgcgacctgaactcctgcagcatgcctctgggcatggaaagcaaggccatcagcgacgcccagatcacagccagcagctacttcaccaacatgttcgccacctggtccccctccaaggccaggctgcacctgcagggccggtccaacgcctggcggcctcaggtcaacaaccccaaagaatggctgcaggtggactttcagaaaaccatgaaggtgaccggcgtgaccacccagggcgtgaaaagcctgctgaccagcatgtacgtgaaagagtttctgatcagcagctctcaggatggccaccagtggaccctgttctttcagaacggcaaggtgaaagtgttccagggcaaccaggactccttcacccccgtggtgaactccctggacccccccctgctgacccgctacctgagaatccacccccagtcttgggtgcaccagatcgccctcaggatggaagtcctgggatgtgaggcccaggatctgtactgatga

SEQ ID NO: 17 - DNA, 1272 bp, Artificial Sequence
  FIX
atgcagcgcgtgaacatgatcatggcagaatcaccaggcctcatcaccatctgccttttaggatatctactcagtgctgaatgtacagtttttcttgatcatgaaaacgccaacaaaattctgaatcggccaaagaggtataattcaggtaaattggaagagtttgttcaagggaaccttgagagagaatgtatggaagaaaagtgtagttttgaagaagcacgagaagtttttgaaaacactgaaagaacaactgaattttggaagcagtatgttgatgtaacatgtaacattaagaatggcagatgcgagcagttttgtaaaaatagtgctgataacaaggtggtttgctcctgtactgagggatatcgacttgcagaaaaccagaagtcctgtgaaccagcagtgccatttccatgtggaagagtttctgtttcacaaacttctaagctcacccgtgctgagactgtttttcctgatgtggactatgtaaattctactgaagctgaaaccattttggataacatcactcaaagcacccaatcatttaatgacttcactcgggttgttggtggagaagatgccaaaccaggtcaattcccttggcaggttgttttgaatggtaaagttgatgcattctgtggaggctctatcgttaatgaaaaatggattgtaactgctgcccactgtgttgaaactggtgttaaaattacagttgtcgcaggtgaacataatattgaggagacagaacatacagagcaaaagcgaaatgtgattcgaattattcctcaccacaactacaatgcagctattaataagtacaaccatgacattgcccttctggaactggacgaacccttagtgctaaacagctacgttacacctatttgcattgctgacaaggaatacacgaacatcttcctcaaatttggatctggctatgtaagtggctggggaagagtcttccacaaagggagatcagctttagttcttcagtaccttagagttccacttgttgaccgagccacatgtcttcgatctacaaagttcaccatctataacaacatgttctgtgctggcttccatgaaggaggtagagattcatgtcaaggagatagtgggggaccccatgttactgaagtggaagggaccagtttcttaactggaattattagctggggtgaagagtgtgcaatgaaaggcaaatatggaatatataccaaggtatcccggtatgtcaactggattaaggaaaaaacaaagctcacttaa

SEQ ID NO: 18 - DNA, 1401 bp, Artificial Sequence
  FVII
atggtctcccaggccctcaggctcctctgccttctgcttgggcttcagggctgcctggctgcaggcggggtcgctaaggcctcaggaggagaaacacgggacatgccgtggaagccggggcctcacagagtcttcgtaacccaggaggaagcccacggcgtcctgcaccggcgccggcgcgccaacgcgttcctggaggagctgcggccgggctccctggagagggagtgcaaggaggagcagtgctccttcgaggaggcccgggagatcttcaaggacgcggagaggacgaagctgttctggatttcttacagtgatggggaccagtgtgcctcaagtccatgccagaatgggggctcctgcaaggaccagctccagtcctatatctgcttctgcctccctgccttcgagggccggaactgtgagacgcacaaggatgaccagctgatctgtgtgaacgagaacggcggctgtgagcagtactgcagtgaccacacgggcaccaagcgctcctgtcggtgccacgaggggtactctctgctggcagacggggtgtcctgcacacccacagttgaatatccatgtggaaaaatacctattctagaaaaaagaaatgccagcaaaccccaaggccgaattgtggggggcaaggtgtgccccaaaggggagtgtccatggcaggtcctgttgttggtgaatggagctcagttgtgtggggggaccctgatcaacaccatctgggtggtctccgcggcccactgtttcgacaaaatcaagaactggaggaacctgatcgcggtgctgggcgagcacgacctcagcgagcacgacggggatgagcagagccggcgggtggcgcaggtcatcatccccagcacgtacgtcccgggcaccaccaaccacgacatcgcgctgctccgcctgcaccagcccgtggtcctcactgaccatgtggtgcccctctgcctgcccgaacggacgttctctgagaggacgctggccttcgtgcgcttctcattggtcagcggctggggccagctgctggaccgtggcgccacggccctggagctcatggtcctcaacgtgccccggctgatgacccaggactgcctgcagcagtcacggaaggtgggagactccccaaatatcacggagtacatgttctgtgccggctactcggatggcagcaaggactcctgcaagggggacagtggaggcccacatgccacccactaccggggcacgtggtacctgacgggcatcgtcagctggggccagggctgcgcaaccgtgggccactttggggtgtacaccagggtctcccagtacatcgagtggctgcaaaagctcatgcgctcagagccacgcccaggagtcctcctgcgagccccatttccctag

SEQ ID NO: 19 - DNA, 6675 bp, Artificial Sequence
  FV
atgttcccaggctgcccacgcctctgggtcctggtggtcttgggcaccagctgggtaggctgggggagccaagggacagaagcggcacagctaaggcagttctacgtggctgctcagggcatcagttggagctaccgacctgagcccacaaactcaagtttgaatctttctgtaacttcctttaagaaaattgtctacagagagtatgaaccatattttaagaaagaaaaaccacaatctaccatttcaggacttcttgggcctactttatatgctgaagtcggagacatcataaaagttcactttaaaaataaggcagataagcccttgagcatccatcctcaaggaattaggtacagtaaattatcagaaggtgcttcttaccttgaccacacattccctgcggagaagatggacgacgctgtggctccaggccgagaatacacctatgaatggagtatcagtgaggacagtggacccacccatgatgaccctccatgcctcacacacatctattactcccatgaaaatctgatcgaggatttcaactcggggctgattgggcccctgcttatctgtaaaaaagggaccctaactgagggtgggacacagaagacgtttgacaagcaaatcgtgctactatttgctgtgtttgatgaaagcaagagctggagccagtcatcatccctaatgtacacagtcaatggatatgtgaatgggacaatgccagatataacagtttgtgcccatgaccacatcagctggcatctgctgggaatgagctcggggccagaattattctccattcatttcaacggccaggtcctggagcagaaccatcataaggtctcagccatcacccttgtcagtgctacatccactaccgcaaatatgactgtgggcccagagggaaagtggatcatatcttctctcaccccaaaacatttgcaagctgggatgcaggcttacattgacattaaaaactgcccaaagaaaaccaggaatcttaagaaaataactcgtgagcagaggcggcacatgaagaggtgggaatacttcattgctgcagaggaagtcatttgggactatgcacctgtaataccagcgaatatggacaaaaaatacaggtctcagcatttggataatttctcaaaccaaattggaaaacattataagaaagttatgtacacacagtacgaagatgagtccttcaccaaacatacagtgaatcccaatatgaaagaagatgggattttgggtcctattatcagagcccaggtcagagacacactcaaaatcgtgttcaaaaatatggccagccgcccctatagcatttaccctcatggagtgaccttctcgccttatgaagatgaagtcaactcttctttcacctcaggcaggaacaacaccatgatcagagcagttcaaccaggggaaacctatacttataagtggaacatcttagagtttgatgaacccacagaaaatgatgcccagtgcttaacaagaccatactacagtgacgtggacatcatgagagacatcgcctctgggctaataggactacttctaatctgtaagagcagatccctggacaggcgaggaatacagagggcagcagacatcgaacagcaggctgtgtttgctgtgtttgatgagaacaaaagctggtaccttgaggacaacatcaacaagttttgtgaaaatcctgatgaggtgaaacgtgatgaccccaagttttatgaatcaaacatcatgagcactatcaatggctatgtgcctgagagcataactactcttggattctgctttgatgacactgtccagtggcacttctgtagtgtggggacccagaatgaaattttgaccatccacttcactgggcactcattcatctatggaaagaggcatgaggacaccttgaccctcttccccatgcgtggagaatctgtgacggtcacaatggataatgttggaacttggatgttaacttccatgaattctagtccaagaagcaaaaagctgaggctgaaattcagggatgttaaatgtatcccagatgatgatgaagactcatatgagatttttgaacctccagaatctacagtcatggctacacggaaaatgcatgatcgtttagaacctgaagatgaagagagtgatgctgactatgattaccagaacagactggctgcagcattaggaatcaggtcattccgaaactcatcattgaatcaggaagaagaagagttcaatcttactgccctagctctggagaatggcactgaattcgtttcttcaaacacagatataattgttggttcaaattattcttccccaagtaatattagtaagttcactgtcaataaccttgcagaacctcagaaagccccttctcaccaacaagccaccacagctggttccccactgagacacctcattggcaagaactcagttctcaattcttccacagcagagcattccagcccatattctgaagaccctatagaggatcctctacagccagatgtcacagggatacgtctactttcacttggtgctggagaattcaaaagtcaagaacatgctaagcataagggacccaaggtagaaagagatcaagcagcaaagcacaggttctcctggatgaaattactagcacataaagttgggagacacctaagccaagacactggttctccttccggaatgaggccctgggaggaccttcctagccaagacactggttctccttccagaatgaggccctggaaggaccctcctagtgatctgttactcttaaaacaaagtaactcatctaagattttggttgggagatggcatttggcttctgagaaaggtagctatgaaataatccaagatactgatgaagacacagctgttaacaattggctgatcagcccccagaatgcctcacgtgcttggggagaaagcacccctcttgccaacaagcctggaaagcagagtggccacccaaagtttcctagagttagacataaatctctacaagtaagacaggatggaggaaagagtagactgaagaaaagccagtttctcattaagacacgaaaaaagaaaaaagagaagcacacacaccatgctcctttatctccgaggacctttcaccctctaagaagtgaagcctacaacacattttcagaaagaagacttaagcattcgttggtgcttcataaatccaatgaaacatctcttcccacagacctcaatcagacattgccctctatggattttggctggatagcctcacttcctgaccataatcagaattcctcaaatgacactggtcaggcaagctgtcctccaggtctttatcagacagtgcccccagaggaacactatcaaacattccccattcaagaccctgatcaaatgcactctacttcagaccccagtcacagatcctcttctccagagctcagtgaaatgcttgagtatgaccgaagtcacaagtccttccccacagatataagtcaaatgtccccttcctcagaacatgaagtctggcagacagtcatctctccagacctcagccaggtgaccctctctccagaactcagccagacaaacctctctccagacctcagccacacgactctctctccagaactcattcagagaaacctttccccagccctcggtcagatgcccatttctccagacctcagccatacaaccctttctccagacctcagccatacaaccctttctttagacctcagccagacaaacctctctccagaactcagtcagacaaacctttctccagccctcggtcagatgcccctttctccagacctcagccatacaaccctttctctagacttcagccagacaaacctctctccagaactcagccatatgactctctctccagaactcagtcagacaaacctttccccagccctcggtcagatgcccatttctccagacctcagccatacaaccctttctctagacttcagccagacaaacctctctccagaactcagtcaaacaaacctttccccagccctcggtcagatgcccctttctccagaccccagccatacaaccctttctctagacctcagccagacaaacctctctccagaactcagtcagacaaacctttccccagacctcagtgagatgcccctctttgcagatctcagtcaaattccccttaccccagacctcgaccagatgacactttctccagaccttggtgagacagatctttccccaaactttggtcagatgtccctttccccagacctcagccaggtgactctctctccagacatcagtgacaccacccttctcccggatctcagccagatatcacctcctccagaccttgatcagatattctacccttctgaatctagtcagtcattgcttcttcaagaatttaatgagtcttttccttatccagaccttggtcagatgccatctccttcatctcctactctcaatgatacttttctatcaaaggaatttaatccactggttatagtgggcctcagtaaagatggtacagattacattgagatcattccaaaggaagaggtccagagcagtgaagatgactatgctgaaattgattatgtgccctatgatgacccctacaaaactgatgttaggacaaacatcaactcctccagagatcctgacaacattgcagcatggtacctccgcagcaacaatggaaacagaagaaattattacattgctgctgaagaaatatcctgggattattcagaatttgtacaaagggaaacagatattgaagactctgatgatattccagaagataccacatataagaaagtagtttttcgaaagtacctcgacagcacttttaccaaacgtgatcctcgaggggagtatgaagagcatctcggaattcttggtcctattatcagagctgaagtggatgatgttatccaagttcgttttaaaaatttagcatccagaccgtattctctacatgcccatggactttcctatgaaaaatcatcagagggaaagacttatgaagatgactctcctgaatggtttaaggaagataatgctgttcagccaaatagcagttatacctacgtatggcatgccactgagcgatcagggccagaaagtcctggctctgcctgtcgggcttgggcctactactcagctgtgaacccagaaaaagatattcactcaggcttgataggtcccctcctaatctgccaaaaaggaatactacataaggacagcaacatgcctatggacatgagagaatttgtcttactatttatgacctttgatgaaaagaagagctggtactatgaaaagaagtcccgaagttcttggagactcacatcctcagaaatgaaaaaatcccatgagtttcacgccattaatgggatgatctacagcttgcctggcctgaaaatgtatgagcaagagtgggtgaggttacacctgctgaacataggcggctcccaagacattcacgtggttcactttcacggccagaccttgctggaaaatggcaataaacagcaccagttaggggtctggccccttctgcctggttcatttaaaactcttgaaatgaaggcatcaaaacctggctggtggctcctaaacacagaggttggagaaaaccagagagcagggatgcaaacgccatttcttatcatggacagagactgtaggatgccaatgggactaagcactggtatcatatctgattcacagatcaaggcttcagagtttctgggttactgggagcccagattagcaagattaaacaatggtggatcttataatgcttggagtgtagaaaaacttgcagcagaatttgcctctaaaccttggatccaggtggacatgcaaaaggaagtcataatcacagggatccagacccaaggtgccaaacactacctgaagtcctgctataccacagagttctatgtagcttacagttccaaccagatcaactggcagatcttcaaagggaacagcacaaggaatgtgatgtattttaatggcaattcagatgcctctacaataaaagagaatcagtttgacccacctattgtggctagatatattaggatctctccaactcgagcctataacagacctacccttcgattggaactgcaaggttgtgaggtaaatggatgttccacacccctgggtatggaaaatggaaagatagaaaacaagcaaatcacagcttcttcgtttaagaaatcttggtggggagattactgggaacccttccgtgcccgtctgaatgcccagggacgtgtgaatgcctggcaagccaaggcaaacaacaataagcagtggctagaaattgatctactcaagatcaagaagataacggcaattataacacagggctgcaagtctctgtcctctgaaatgtatgtaaagagctataccatccactacagtgagcagggagtggaatggaaaccatacaggctgaaatcctccatggtggacaagatttttgaaggaaatactaataccaaaggacatgtgaagaactttttcaaccccccaatcatttccaggtttatccgtgtcattcctaaaacatggaatcaaagtattgcacttcgcctggaactctttggctgtgatatttactag

SEQ ID NO: 20 - DNA, 1272 bp, Artificial Sequence
  FIX-Padua
atgcagcgcgtgaacatgatcatggcagaatcaccaggcctcatcaccatctgccttttaggatatctactcagtgctgaatgtacagtttttcttgatcatgaaaacgccaacaaaattctgaatcggccaaagaggtataattcaggtaaattggaagagtttgttcaagggaaccttgagagagaatgtatggaagaaaagtgtagttttgaagaagcacgagaagtttttgaaaacactgaaagaacaactgaattttggaagcagtatgttgatgtaacatgtaacattaagaatggcagatgcgagcagttttgtaaaaatagtgctgataacaaggtggtttgctcctgtactgagggatatcgacttgcagaaaaccagaagtcctgtgaaccagcagtgccatttccatgtggaagagtttctgtttcacaaacttctaagctcacccgtgctgagactgtttttcctgatgtggactatgtaaattctactgaagctgaaaccattttggataacatcactcaaagcacccaatcatttaatgacttcactcgggttgttggtggagaagatgccaaaccaggtcaattcccttggcaggttgttttgaatggtaaagttgatgcattctgtggaggctctatcgttaatgaaaaatggattgtaactgctgcccactgtgttgaaactggtgttaaaattacagttgtcgcaggtgaacataatattgaggagacagaacatacagagcaaaagcgaaatgtgattcgaattattcctcaccacaactacaatgcagctattaataagtacaaccatgacattgcccttctggaactggacgaacccttagtgctaaacagctacgttacacctatttgcattgctgacaaggaatacacgaacatcttcctcaaatttggatctggctatgtaagtggctggggaagagtcttccacaaagggagatcagctttagttcttcagtaccttagagttccacgagttgaccgagccacatgtcttcgatctacaaagttcaccatctataacaacatgttctgtgctggcttccatgaaggaggtagagattcatgtcaaggagatagtgggggaccccatgttactgaagtggaagggaccagtttcttaactggaattattagctggggtgaagagtgtgcaatgaaaggcaaatatggaatatataccaaggtatcccggtatgtcaactggattaaggaaaaaacaaagctcacttaa

SEQ ID NO: 21 - DNA, 34 bp, Artificial Sequence
  pF8_short_XhoI_FOR
cagcctcgaggagctcaccatggctacattctga

SEQ ID NO: 22 - DNA, 33 bp, Artificial Sequence
  pF8_AgeI_REV
cgaaccggtgacttattgctacaaatgttcaac

SEQ ID NO: 23 - DNA, 36 bp, Artificial Sequence
  pF8_ECL_XhoI_FOR
cagcctcgaggtttttaaaacaatagttgcctaacc

SEQ ID NO: 24 - DNA, 33 bp, Artificial Sequence; identical to SEQ ID NO: 22
  pF8_AgeI_REV

SEQ ID NO: 25 - DNA, 29 bp, Artificial Sequence
  pF8_enhancer_Short_MfeI_FOR
cttcaattgggggctcgctcgctcagtac

SEQ ID NO: 26 - DNA, 29 bp, Artificial Sequence
  pF8_enhancer_MfeI_REV
cttcaattgctcaactcctatggtgccac

SEQ ID NO: 27 - DNA, 29 bp, Artificial Sequence
  pF8_enhancer_Long_MfeI_FOR
cttcaattgtcgccaccacttggcttccg

SEQ ID NO: 28 - DNA, 33 bp, Artificial Sequence
  pF8_Long_XhoI_FOR
cagcctcgacgacgagttcccacaaacgttacc

SEQ ID NO: 29 - DNA, 19 bp, Artificial Sequence
  DENV RF2_FOR
gacccacctcccaaccccg

SEQ ID NO: 30 - DNA, 22 bp, Artificial Sequence
  GFP_REV
cgtcgccgtccagctcgaccag